European Patent Specification EP 3 548 636 B1, published August 9, 2023. Title: METHOD. Applicant: Oxford Nanopore Technologies Limited. The sequence listing filed with the application follows.

SEQUENCE LISTING (46 sequences)

SEQ ID NO: 1 - DNA, 40 bp, Artificial Sequence
  Control Adapter NB01 (barcode top strand)
aaggttaacacaaagacaccgacaactttcttcagcacct

SEQ ID NO: 2 - DNA, 45 bp, Artificial Sequence
  Control adapter NB01 (barcode bottom strand)
ggtgctgaagaaagttgtcggtgtctttgtgttaaccttagcaat

SEQ ID NO: 3 - DNA, 59 bp, Artificial Sequence
  Follow-On Adapter (barcode top strand)
ggcgtctgcttgggtgtttaacctttttgtcagagaggttccaagtcagagaggttcct

SEQ ID NO: 4 - DNA, 64 bp, Artificial Sequence
  Follow-On Adapter (barcode bottom strand)
ggaacctctctgacttggaacctctctgacaaaaaggttaaacacccaagcagacgccagcaat

SEQ ID NO: 5 - DNA, 59 bp, Artificial Sequence; identical to SEQ ID NO: 3
  Follow-On Adapter (barcode top strand)
  misc_binding (23)..(24): nucleotides separated by 4x iSp18

SEQ ID NO: 6 - DNA, 64 bp, Artificial Sequence; identical to SEQ ID NO: 4
  Follow-On Adapter (barcode bottom strand)
  misc_binding (35)..(36): nucleotides separated by 4x iSp18

SEQ ID NO: 7 - protein, 262 aa, Escherichia coli
CLTAPPKEAARPTLMPRAQSYKDLTHLPAPTGKIFVSVYNIQDETGQFKPYPASNFSTAVPQSATAMLVTALKDSRWFIPLERQGLQNLLNERKIIRAAQENGTVAINNRIPLQSLTAANIMVEGSIIGYESNVKSGGVGARYFGIGADTQYQLDQIAVNLRVVNVSTGEILSSVNTSKTILSYEVQAGVFRFIDYQRLLEGEVGYTSNEPVMLCLMSAIETGVIFLINDGIDRGLWDLQNKAERQNDILVKYRHMSVPPES

SEQ ID NO: 8 - DNA, 16 bp, Artificial Sequence
  Morpholino oligo
ggaacctctctgacaa

SEQ ID NO: 9 - DNA, 17 bp, Artificial Sequence
  Tether
  misc_binding (2)..(3): nucleotides separated by 4x iSp18
ttttgaccgctcgcctc

SEQ ID NO: 10 - DNA, 12068 bp, Artificial Sequence
  Basecall_Alignment_template 90e5fe72_read_ch2_file10
tggtttgtcagagaggttcaagtccagggttccttgcctgtcatctatcttcggcgtctgcttgggtgttaacgcctctgcaccggacggtcccctcgcccctttgaggagggttaggaagagaaaaccgcacctgtaccggatcggttatttcgcattcttatcagacccactgcaaccgctgaatatgcaggcataacaggtgcaggatcaccaggcaatgcagcaggtaaatatcattgccgtcccagactttggtggtgaccttattgtccacgtccagctcctgccaccgggaaccatttcatagtccatccaggtacttatgcagtactctcccaccatgtttgataccaggtttccttggcgatcgccagtattgacggtgtaaacgcgtaggccgtacccattgcttcgacgataggccagcgtacacgttcgcggaccaccggtttccttcccagtcaacgacataaacggctccgtccgcgccatcggtgcccaggcatcgcgcacggtggcgttaaacgaacctttggcatcttctagcaacctgctggtggttgttcgcaacgggcttcccagggccatatggatgtacggcggcattaaacggccccattcgatccggtggcctggtgcactcgggcgcgcggaagcgatgcgccgggttatctttgttgtaatcccggcagccggattccactgggtatcagtgttcgtgctgcccgataatgattatttctggcgacatcgtggatgtcacggaagccacgcgaatcgcgcgatcagccattttgtcggtgacgtcataaacaatcgaagcttccaccgcgtgcatattggcattgccgccgcggtactcttcgattttctgaaggcttcgtcccgggattcaggcatatcttcttctccagaaatatttctcgataatttcgtatgggccttaatcagtagcgcgcttccaggtgaccgtttggcgacggcgctggcggcacccagcggaaacaaagtgttagtaagccctgttgcaggcatccaccacgccctctgatgccgttcgcacgcggcgtaccagccgccataattttatccgcaccatcgccgttcatggctttgatgccgtgatcaaccaacgatggcgccaggtcagcccatcgccgcaaccagcgatcgcgtgcaacatacgagcggtgatccacagatgggtgcccatctcttctttgatttgccctttgtgcctaaccagccatgcagtcggcactacggaattttaccaaaatcaaagatgcggtcggtttcctgttcagccaacggttggcagcagggtgttaaaccatttcattcataccatctcatcttggcggcgtttagccatcatttcgtcgacgatatcgccaagttgttgtaatttctgattacaaacgtcacgcagcatcagctcgttgtctggtaaaccgacgaccgtcttgaactgcacggcctgccaggaatccccgataacccaccgtcgttactgccacgcgtacgacgcaggaacgatttttcgtcgacaccgaagagatctcacccatggcgccattaatgctgtcattcagacgttgtgaagcacagaaagctcttgttgcggacctttgccataaagcggcattttcagctttgtgaaggtcagcgccactttctcgcccggctctttgagcacggcatcgatgatcagcaaccgcgatcgaatttatgctcacggcacaacggtgggcggacgctggttcgtgatgcttaccagaccgtgagtggcacagttcgttgaactctttcaccatatcgaagacgttgctgcgcatcttcatcactacgccacagcaccagcagttttaggctttgccaccgtcttgtttgatcttgtggattgattttgcggtcagcaaccacgctatcgtggagattcgttctgggaatgaactttcatcggcggcgaccgcaatcatggcgcaactttgtaatcgcattttgctcaaccacctggcggtaaccgtgacgatctaccaagtccttgagcataaggcgaagacgcgccgccggcgttaacacgaaatccagttaaaacgctactcctgagcttctggaagggcggtgccccagccgcggcaaacatcatgcacgctaaacttctgcgctgatcgacctgctgcgtagcaaaaccgccgatgcgcgtaatgtcgttgatggtgtgcttattcattcatttattccttttatccgatcgttacattttactttggcagtcatcccagcgcgacacggacctgttcaagaatggcggaccgatctggcgacccgcgacccgctgcgcgcctggctataaacctcccatcgggcagcccagcggcattggcacatgcagctggttggcgacatcaagggcgatgcaagattcttctgggcaagatcgatcatgaaggcgggaaaagatctccgctgaggactttgtttggccaggaagtggtgaagtgacctttaccggcagcatttgctttcatcgcgacggcaacatcgaggaagttagggcttcgcacaaacggcaacttctgccgaaagcacgccaggcgcaatgcctcgccagttgttgatgagcaacgcggatccccatgcccggaccgccagcgttgatcaactcactgccgctcaccatcggatcggtgtggcacgtccaactgttcaacggtgccgccagccagccagtaacagagtaccggtaatggcatttgcagaagtacggcctaccggtgggtgtcatcatactgaaactgcggcaccatcggcaatcaattcggttttgcagcggatggatggtggacatatcaatgaccaacacatggtgataaagccttcgcaaaacgccgtttcaccgaacaacacgttgcgcaccagatcgccattcggcaacatggtatgataaattcggcatctttagcggcctgccggttggcggcggggtcacgctgtctaccagatactacaccttcggcgttcacatcaaagacgcgaagttgatgcccttgctgcaataaattgctcaccggtggcggaccatttgtcctaaaccgataaacgcgattgctgccgcaaccctcctcctagaatatggtgtgctcacttttgtcatttatgacatgctttgcttgtctgttttgatcgtatttgtaatttatcgtcaagattgacagccgtcaccccaaacaattggtgaggtggtagacgcatcccaaatcactgagaatgaccatgattcattgttgccaatggccaagtaccaaccgtgatggatcgcatctattacgtggaaggaataccgacggagagcgtgaaaccgtggcgaggtatactggagagttggtggcgggccagcggcgacggcggcggttgcggcagcaggctgcgaggcgcaaggtcatttattggtcacgtgggtgatggcggctggtggcaacctgctggcagagctggaatcctgggcgttaacacccgttacgcaaacgagcataaccaggcgaaatattgcaatcaccatcatggtggatacaaggcgagcggataatcattaactacccccatgccggatcctgctgcctgacagagtggttggagaattgatttctctccggtgggatgttggctggcagatgtacgctggcacgacgagcgctaaaagccttcgccctggccgtcaggcgggtgtgatgaccgttctggacggggacgatgcgccgcaggaccatccggtgaaactggtggcattaagcgatcacgcggcctttcagaaccggtctggcagcaacgggcgtgaagatggcttggtgcgctaaaacaggcacaaacgctctaaatggtcatgtctatgtgaccagggtagccgcgagctgcgatagctggaaaatggtgggcgtcgcatcgtagccttcaaagttgatgtggtagataccacaggtgcgggtgatgttttcacggcgcgcacagcggtggcactggctggcaacaagtggggatttagcgagtcggtccaactacgtaacagtgtggcaacgttaaaatacgtcggtggacgaccgggatctgactgtgatcaaacccgatctttgtcacttttgtatgaaatgccaggggtgatggtttcgaggaattttcgcaggccttaccgaactaaccggtaacccgcagcgaccaactcctcctgctgatcgccgagcgggtatatgaatattgatgagctggcaaatcgctggatgtctccacacagacggtccgcgggatattcgtagtcatgagcaggctgattacgcactgcagctcacggtggcgcggtcagctcgcatcagtgtgacgttcggcagcgtgaggtttcgcaagctcgagaaaaacgttgccgaagcggtggcgaactatattcctgatggttcaacaatatttatcaccagtggtacggcttctattcgacgtatttgcccaggcgttgccaaccataatcatttacggataatctaccagcttgaagcctcgtgtggcgcatattgctacaacccgcgctttgaagtggtgcccggcggtacgttgcgctctcgccaatggcgggatcattggccttccggcggcgtcgctgtggccgatttcgtgcgcgattatcggtaacaagcgttgccggccggtgagcgatggcgcgttgatggagtttgataagcagaaactaacggctgggtgaaaacgatgatggcgcacccgaaatattctggtcgccgatcacacaagtatcatgccttcggcagcggttgaaattgataacgtggcacaggtcactgcgctcttaccgacgagctgccgcccgctgcgctaaatcacgcttacaagacaataggtaaatcattcttccccaggagagacgcgcgttacgaccgttaacctggccataccttgccacaacccaaacccatcctttccactacagttaatttcttgtggcgcgaaagacacaaatactctatatctttgatttgagtaatgtgattatcaatgtcaacaccaacgtgtgctggggcctgggcgattgcgcatgttacttcagcatcgcttaagaagagtttattgctgggagcgtttcatctggcatgggcattgaaattagcgacaagcgttcacagagagcgctgtatgtctgaatggctctaccactaagctacgacagttctctcacggctggcgacagtgtttgttgcgctacgccggaagtgatcgccgtaatgcataaactacctgcgtgacaggggcatcgtggtggtgctttccaataccaacctgcataccaccttctagcccggaagaatacccgaaattcgtgatgctgctattatatctatctgtcgcagatctggggatgcgcaaacctgaagcacgaatttaccagcatgttttgcaggcggaaggttttcacccagcgatacggtctttcgacgataacgccgataatatgaagggcaatcaactgggcattaccggtgttcggtgaagataaaccaccatccaagctatttcgcagtgttatgtaaaaaccattcaggacaaaactaaggcaccatgccatccactattgggcctggcacaaaactactctggcagcacgtattgaggacaacatgacaacctggcggtaaccttgcctatgcatttatgctctcggctaattcgccgctggttgccgttgttttgcgcttttcgccgcttttcccatgttttccgacgtcagcattcagttacgtcactttattattttgtaactttctgcctgctgcagcgatgttattcagcggtatatgaacaatttgttgccaattcaacaagatgaccgccgttggggctgatgggctgatcgtcaccgcgttattgttgatgtactccatccgatagcgcgttgaataccatctggcgcagtaagtaagcgcgaccaaaatttactcgttcaccgtcactggtggattttaacactaaagacccgcttctggcaagggccagtctggcgatcagttcctgttgctctccctgcgctgggcgaaacgtctcgctctgtcatcgataacgtgcgtatttttcccgttgctgttgtcgtggatctctccttctggttgccagctggcattgttctaccatccgtacctaaccgcggcgcgattgtcagcgtttgtcgccacactcctgttcgaagcaggaaaggtttcgcgcatatctacatgttcccgtctatcagctcatttatggtgtgcggcggtgatccccattctttgtttgggtctactggacatggtgtatcgtcttcgcagcgccgaagtactgtcactctcgggaataccgcaaaagctaaaacaagcagcttcgacaagaagacgacgaaccatgattgcattaattcaacgcgtaacccgtgccagcgtcaccgtggagagaagtgggcgagggagtagctgggactttgcggtgttattagcggtgctcaaaggtgtgaacgaaagcaaaccatctgtgcgagcattaacagctaccgcatctttatgatgcgaggcagatgaatctccagcgatgcaacgggcggcggcagtgtgctggtggtttcccagtttaccctcgccaccagatattctgaacaggggatacttaagtttctctcaggtgcatcacggatcgcgcagggcgttatatgactatttcgtcgaacgctgccgtcggcaagagatgaacacaccgacaggccgcttcgctgcggatatgcaggtatctggtcagccggccagccccatgtgacattctgtgatttgcagtgctgagccagcttccggtttgtcacgggaaacgaaagtatcgctatgtatctgccaggttccacaaacagaagaagaattgagagcgttactatcagtttcgctggaaatgttgcgcccttcatcaacaggttcggaacacgcgcgtgggatgcgatggcgcatcgcagatggtcacgtcgacgacagggtaatctcggtaacggtaaactgcgactgtatattgtctaccgacaatgaagcgtccattcaacatggccgttcatcccggcgtgcgggacaagggttaggcgctgatggcgatgaccacaggtcggtggcgcgtcaggaagagcgttaagcgcatgactaacagcgcccgtgaagacgcggtgcggagttttcgccagcgggtttgtgtcagggagaaatcaccacataaccacgccgattcgccatttttgatgattaagcccgtcgcctcgttgacattcaccgcatcgcggcgactggtgcgcctggctgtgggcggtacgaacatatcgcgggtgaaaaatgggcgtgcgcattcagcaatataccgggcaaaatttatcactaccatgccgaaaccggcaatcaagtccgcaccatacgctgtttaccgaagacatttctcggcgacgctcactggactggggacttatctgtgatacgcgtgaacgccacctcggcgaacgattattcttgcggatacgcatatccacttcaaccagccgattggcggtaaacctcgtgcggtacgccgacctcggtatacgcaagcggcgatctcgaccgtcgcgcgcggacgaaagcaggtgcagatgcaggtcgaaatctttggcaacagggctaccgggtgcagtgtttgaaggcacgtatgtcgttctgcttgcccgcgaaagccatttggcccgtatgaaggcgggcgagtagctgatggaaggcgaacacctctctctcttcaggtgcattatgatagatcgccaagctatttcagttgctgtaaataagaactctataagttacgcattcttcttcgttggctccatgcggtgtcttgccacatcactgttcaggagcatttaaataatactttagcgaactggtggcaattatcacgccgaatagcgcttattccatcatcttagttcatgtttgagcgatttttgatagtcaaaaccccactctggtgccatacttttctcttaaatactttaaaatctatagctaacaaacaatatacaaagataatggatagctcgtcagtatcaaccatttaccctttcttgtgttatgaatattatgttgtatgtttgctcttaaaccgtgggaaggaggctataatggttgccaatataatctatttctgtgaaagttattctgttgttaatttgaaaacaactttcccagactgttaccaacaaaattatatgatgaacaagtaaagaccggttggtggcagtactacaaccgatgcgatgaagattaatttcaccgccaaatcctggtgctgttaggatgctggcgttttcggctacaccattcaagattatgcaaataatatctcagaccaacaatatattcttaacacccataattcatctgagcgatactaaaccattttgagtaataagtaaacagctacagcactcttattatttctggaaaacgcctcgcaaaaacaaaacataaaatccgctttttaaatgattttccggcgccattttcgcgccacattaatgagtaatataatgagtattagtaatgtgtgtatgcggttttcttcatttacatcgaagaaccgttaaacggctgaacaagcttcggggctggcgtaaggtttctgatcaatttacgcgaagcggtagagcaatatctggaacgtcagcaattcccgaatacgtaaaacaaaggagagcaggcaaaagggaggtagttggtgttgatgatcgttaggagcataagggaatgacaagaattttgttcttgaatataaaaacagatgcccttattctggtattaatgaggctgtttgcgaacttataataactgcaactgttacatcatatctggaaacgcctcgcaaataaaaatgatgcaataaatagagctttcttcaagattcggcaaggtacttttctctccatgtggattcaaaatgatattggcggtgttatgaactctctggcagtacagatatgggcgggaattttactcgatttatcgaatggggtgattcaaagcaacttgatgatctcgaaggtgcagcgcaatgtttcctcgtgcggacctattaagggaagcggtagatcatacctgataatcaaatcaaacaagcaagaaccaatgttcctggcatctggcaaggaaggtgcagaagatgattatcgaatatcggcgtaagctgcgcgagaatggtgtgggaaaatgatgtcaatcagattgctgacaacgtgcccgttgttcgaaatgccggatgcggcgtgaacgccttatccggcctacaaagtcagtataaattcaatgtattgcagtttattggtaggcctgatggctggcgcatcaggcaatcttgctgtcatcggtctcatgcccataaccttattgatgtgggtggtgggtaaattggtaaaccggcactggcggcatggcggtgttaacgcggaatacgagatggtgtcgtcaccacctaacgagctgtaatccgggcgacctgcgccaccggaaaacgtcggggtactcttcacccggaaacaggaacgggttgatggaatgcgaactcttcttcttgtattcgtgcgtccaaagtaccaagaggcgaaggtcatctactacggcttcgttttggtctttttcctgataagaaggtactggtagtgtcgctggtcatcgcagctttctggctttaatgcccggcctatttcgtcatcagcagccagtattacggtttgccgctctctgcggattgctgcattcccgcgcactacgtgccattcagtttcacgggttacggtgcagtaacaccttcggtggtgccaatttgcaccatgctggacttcggcagcagaaccacaaaccgggcaatattgacgttgctcgccaaacattcagcgcgggctttgccggatcaggtcggccatgcgcccggtaggcgacagtgcagccagataaacggcgctttatcgctgctgacggacgagaaaatcaggagcaaacagcgcgctggccatatcttccagctcctgagtcattaccttctccagattctcaatcactgccaccagcgccgggccgctcatttcaggtttcagctcggcaatcagcgccatcaagcagctttccggtgcttatcgcacggcaggcggaatatccagcgggcttgccttgtgcgctggcttctttaatgcgcctgcagtcagatccatctccagcgcacgatttgttcgtacagcaccacttcctgggcggtaaggcgtcagctttgtaaagcgcaggtaatcgcagaggatttattttctgccagctcgcgcagacgctcggcgcggcggttgtataaattcttgagccgaggaacaataacggcggaatcgcatatccaccgtacgtttctcgcgaacccagctcatcttgcggattatgcgaatattcagctctttccgttgtcttgcagttccgcattttctgctgccgggtgatgtttcttcgccctggcattgtatccttccaccatggcattgtcgtgcctttcacccaagggtgaatgccaccatgataaccctgaataacgccacctgcggcaaatagatgcaacacgtgctgtagaatcggatcaccggattgaaagcaaggcgcaaaataaggacgccagataatcacgcgctcgcagcagcagaaccgggaaaataatcgcaccgcccgaagaaacgcatttcggccgaagttataacgcccgtatactcacctcctcgttgacgacgatcttacgaatattcttcttcaaaagatagcatcatccccgattgattggttgtgatgcccagtaacggaaaaacggtgatgaaccctgagacaaaacataaaccacgcaccgacaaacgggtgcagaattctacatatacagctgcgaataccgcggttgcatcaaccagttgaaggacggggcaaaagccgctcaccgccgccggggatgaagcggccacggtgatccagtggttgatacgttccagcgcggtgcagcgcacggtggtgtcgtcgtttcatttgcgctctcgtcttctcttcgtgcagattattctcttcctcatcaccacggttcaggccgacaccccatagtagaagatactggccgcaagggccagccgcaaaataacagccgcgagcggtttcagatgcctttcagaatttgcggtttcttcccggttcgggttctccggcaaaccatgatactgaatttggcttgtcaacgtggtgcaacacattacgtgtactaccgacataccggatcgtacagacccacattgtcgtaaccaccaggttttcagctcagcaacgcgctcgctctttccaacgttttcatcaaactcgtacaagtgaatccgcgcccgttgggcaggtcttcacctgagctgaagttctaccaaccaccgcacggatcgacgcagcgtacattggcgaacacggttgtcagcgcaggtttgagcgcggggtaatgaacggacagcctggtacatgccaccaaccaatgcactgctcggctgaagtcgacattaccgttgacacctgaataattgcacgctacaccaggcacgccttcaggcagcctggatggaacagtacgccacagccgtctttgcggatcaaagccattcagtttgtctggctgtccacttcgagcgcattaccgtccacgatttggcgctaaatcattggggttgtcgtacaccccaatgttattgccgacattgtatcgcagtgtcgttccctctgaacacgccaccacaaccgggctttacagccgatacaggtggtaacgtcgatgagtttcgcccacttcttcctggaagtcccgcgcctgaggcgcggggtcgaacattagtcgcggaacgacgaataagttaaacatgacagacgccgagatagagcgacgagcaaagtaaggaaccccgcctctctgacttggaacctcgttccagcagtacagccaacttg

SEQ ID NO: 11 - DNA, 11605 bp, Artificial Sequence
  Basecall_Alignment_template 90e5fe72_read_ch2_file11
cactttgataagaggttccaagtcattcctactgcctgtcgctctatcttcggcgtctgcttggtgtttaacctattcgtcgttccgcgactaacggtctgaccccgcgcctccaggcgcggaacttcagaaaagtggcgaaactcatcgacgttaccaccagctctggctgtaaacccctgtcaaaggtggcgtgttcaagtggaacgacattcgcgaccgtcgtaataacattggggtgtacgacaaccccaatgatttaaacgcaccaaatcgtggacggtaatgcgcgctatcggtgaacagaacgacaaactggaatggctgatccaccaagacggcagcgtactgttcgatcaggctgcctgggcgtgccggcggaagattaccagtgtcagtatggcctcgtcgacttcagtcccaggcggtgcggtggcatgcggattgtgcgacaccgcgggctgtccgttcgacattccgcgcggaagacaaccgcgtctacaatgtgccgctgtgcgtcgaccgcgtggtggttgggcgaaccagcctgcgtgaagaccaccgcgcgggcgcgattcacttcggtacgaaagagtcggtaaacgctggcgaaacgagcgttgctgagctgaaaacccgcggttacgacaatgcgggtctgtacgatccagcgagaacgtcggtggtacgtcatgtacacgtgccgcaccatgctgaaactgaccaaatctgtatcgcgaagcacaggagactaatcagcgaaaccgcaattctggaaggcctcctggaagccgctcgcggctgttggcttgcggctacccttgcggccagtatgtcccgccgtggtgtcggtcgaaccgtgcggatgagaagaaataatcctgcacgagaaagacgggcgcaaatgaacgacgtgacctgtcgtgcgctactgcgcgccggaacgctatccaaccactggatcaccgccttcttcatcctggcggcggtgagcgggctgggctttatttcccgtcccttcaactggttgatccaccaaatcgccatttaccgcaactggcgttctgcacccgtttgtcagcgtggttcatttgcctcgttcatcatcatgttttccgttgccagcatctggcttcatcaatcgggtaatcttttggcgaagaatattcgtagatcgtcgtcaacgaagtaggtgacaccgggcgttataactggtcagaaatgcgttttcctgggcggcgattatttttctggttctgctgctggtgagcggcgtgattatcagcgatcatatttacgcctgctttctccgtagtgatcgattcgcgttaatgctgccattcatttaccagtggcgacagccagcggattatcatggtgcatatctgcgccgccctttgggtgaaaggcacgatgccgccatgaaggatgtaccagcgcctgtgggcgaaacatcgcacccgcgctgatgccgtgaggtccgcaagacaacggaaagccaatcagtattcgcataatcctggaatgagctgggtcaagcggcttgtacggcgagatatgattccgccgttattgttcctcggctcaaaattaaccgcgccgagctgtctgcgcgagctggcgaaataatcctctggtgattacctgcgctttgctgcgcttatcgcccgccaggaaagtggtgctgtacgaccatccactggagatggtctgtgcgcgcataaaagccagcgcacaaggcaagcccgcagatattcacgttctgccgcgtgataagcactggcaaaaactgctgatggcgctgattgctggcgctgaaaccacaaataggcccggcgctggcggtgaagtctggaggcatcgactcagggctggaagaccagcccagcgcctcctgatttctcgtccgcgtccgtgctgataaaacgccgttgtatcctgggctacgcaatcgctctactggctgaatggccaatctcagtcaacaaagcccgcgctgagccacgacgagcaacgtcagccttgcccggtttgtggtttatgccggtgtccaaagcataagttaccgtggcaccactcggaactacgacctgcactgcaactattgtgaaactgaatagcacgtggtgcgcagccatcaacaactgcgagcaggcgacaaacccattaccattcgctggatgacgagcaaacgcgataaagccaaagctgcgtgacgacgcctgaaaattctctatcggaaaagtccagaaatcaagccgtaacgggtggcctcctctggtactggacgcacgaatgggcaagaggctatgcccgcagttccatcaaccgttcacatttccgggtgaaggtaatctcccgacgttttcgggtaacaggtcgcccggattacagcgctcatggggtgtgacgacaccatctctcgtattcgttaccacctcaaactgtgccgccggtgccagtttgactcaatttcaccacatcaataaggaccttggcggggcggtgacaagcgtagattgcctgatgcgctgcgcgcttatcaggcctaccaataaactgcaatacgatgaatttatacgactttggcaaggccagatggcgttcgccgcatccggcatgaacaacgcgttgtcagcaactcgattgacatcattttattgttcctcgcgcaaccccacgctgatattcgacaccatcttcacaccgcctgccagatgccgggaacactggttcttgctgttgcgttgatttatggtgatgatccagcttccttaatgggtccgcacggaagattacatttgcctcgagatcatcgttgtaatcacctcattcgtcgtcaggtaaaattctgcccatatctatacctgccaaagttcaccaatatcacttcaatatcattttgaatctggaaaagtaccctgccgaatctttaaaaactcatttacacttatcattttattttgcgaggcgttttcagatatggtcatggcagttgcggattatattcaagtaaaacaaccttgtattaataccagaataagggcatctgtactatgttcaaaattgaaaattttgtcattccttatgctcttacactgatcatcataccaactacctccccctttgcctgctccttacagcactgggaattactgacgttcagatattgctctaccacttcgcatccattgcagatcgtgaaacccacgccagcaagcgttccgtgttagtgcctcttctgataaatgaaaaaccgtatacatcgccattaataccttgtattactcagccaatgctgtgcgaaagtatggaaaatcatttaagcggattttgcatgttgttttgttgcgaggcgttttccatatgctctatagagtgttgcgttgtttcatttattactcaaatggttagttatcgctaaagtggattatgattactatgaatatattatattcagaatgttgttgcataatctgaatggtgtaactgaaaaacatatcagcatcctaacagcaccggattttaaattgaaattaatctttcatctgaaccggtcagtactgccgcaaccggtctttacttgctctatattctatatttgtggtaatgattcaggaaggattgttttctaaattaacaacagaataactttcttgtttaatgagattaatgtggcaaccattataataccacggtttagagcaaacatacaacatattattcataacatacagagcagtaaatgaatgatactgacaatgatgctagtccattatctttgcataatatttattgctataatttaaaaatatttatgagaaagtatggcacagagaacgactatcaagtatcagcaaactaagatgatggtggcattatctgcgataaaattgccactcagttctacaaataatatttaaatatactgaacagtgatctgtgaacgtaagacccaacgagaataaaaatttatagagttcttgttttaatataacgaaaccgggaccagcaaatgacctgaatagggagaacgcttgcctatgccatcagctactcttcttcgttcctcctcttcttaccgggccaaatagctgcgccaggcgaacgatacgtgccttcaaacagctgcacccggcgtctcgtcgccaagattttcgacctgcatctgccgcggccagcgccgtcgcgcgccagacggtcgagatcgccgctgagcaccgaggtcggctaccgcatgagtttaccgctatcggccttggcggcggttaagccgcatcccatcacgaacaagtcgttccgccggggtgtggcgaccgcagcatcggccagataagtcccaaccagtgagcgtcgccagtgaataaactcccgaaacaaaaccgccgtatggtgcagttcctgattacggttctggcatggtagtgaccgtacgcccggtatgatacccgaatgcgcgccattttcactggcgcggaatatgttcgtaccacgcctgttcgctgcgcgcaccgccgcgatgcggtcatccagagtggcgacgggcttaatcgtggcgaatcggcgtgtggttggcgtggtgatttctcccagtgctcggcaacggcgaaaaactcaccgcgtcttcacgggcgctacaggtcgcacgccaacgccttcctgacgccaccgactccaggtcatcgccatcggcgcccttcatcctgcgtcgggatgaacggccataaagcaaatggacgcttcattgtcggcattaatatacggcctaccgccagattaccctgctcgtcgacgaccatctggtgatgcgccatcgcatcccacgcgtcgcgttcagaaccttttggttgatgcgagcacgacatttcagcagagcctgataacgcatacaattcttcctgcacggaaccgaaggtgatacgccagcgtactctcttgtttcccgtgacgaccctgaaacttcagctcgcctgcaaccaagaatgtcacgggccatcgtgataacgataccctgcatatcccgcagcgaagcgtgtttgcgtgttcatctcttgcggcggcggcgttcgacgaaatagtcatataacgcctctgcgcgatccggtgatgcacctttgggcttgggctttgtcccgttcagtatcacggcgagggctgaaaccaccagcctgccgccgcctgttgcgttgagattcatcttgcttcggcatcgctaaaatccggtatgagcacgtgattctcctttcgacacccaataacaaggtccgcgccaatttcgcccgtcgcctatcctctacatttgggattacgcgttaattaatgcaatcatggttcgtcattcttgttcttcttgctggttgcggtattccccgagtggtaatttcgcgccaagcagacgtacaccatgtcagtgttaaaacgaagagaatggtcaccgccagcacaccataaatgagctgatatgagcggaacatgatgtaaacgcaaacctttcttctgctgattaagtgcggcgacaaaacgcgccaaacgataaatcgcggttaggtacgccggatggtaggaacaatgctgtacagcaaccagagatccccgacaacaggaaaaatacgcagcacgttgtcggtaaccgtattgatcctcgccagcgcaggagaaggcaatgaactgatcgccagactggcccctaccagcattcgcaaatcatccagtacgaacagtaaattttggtcgcgctcgtttaccacgccagatggtattcaacgctatcgatggagtacatcagcaacaataacgcggtgacgtcagcccgcacgccccaacggcggtcatcttgttgggtggcaacaaattgttcgatataccgctggtaacatcgccagtagcaggcgaagttgcttaaagtagtgacggcttgaatgctgacgtcgaaaacatgggaaaagcgacgctttaaaagcaacggcagccagcggcactaatgaacaacgacccttgagcaaggttacctgccagggttgtcatgttgtcctctcaatgcgttggtagtttgctttcgaccttggacgggtacggtgcctggctttgtctgaatggttttaacaacactagcgaaacggtccgggatcaggtggttgctcgctactgatgctggtaatgcccggctgattggctccttctatgacccatcggcgttatcgtcgaaagaccttatcgctgggtgaaaacgccttccgccgcaaacatgctgttaattcagccttttcgggacgcatctagatcttgcgacagatagatatgattgtagcatcacaattttccgggtattctccggcagaaggtggtatgcgagcggttgtggaagcaccacccgcatgatacctgctcacgcagtttgtgcatgatgtggcgatcacttccgggcgcagcgcagcaaacaccgcctgccagccgtgagagagcgctgctcgtagcttggctgagccaaatctcgtgacacagcgcctctgcgaacgcttcgtcataatttccccacactcatgctgatgaaacactaccatatgaaaactcttcttaagcgatgccagcggaatacgcgttgaaatcatcaggctcccaacacggttaaagtcgatatcgacaacattacctaaatcaagatatagagcattttgcctcctttcgcgccacaagaagtgctgtagcaggaaaggatgggtttaactatgtggcaagtgtaaaccaggttaacggtcacaaaatctacgcgtcttcctgggaaaatgatttcgttggctgtctcccaaccgaaaacgtgattttagcgccggcgagcggcaactcgtcggtaagagcgcagtgacctgtgccacgttaccaatttcaaaaacctgccaagcatgatgccgtgtgatcggcgaccagcagggctgttctcgcgtacgccatcatgtttcaccacgccgctgaacacatcaactccatcaacgcgccatcctctaatcgctaaccttacattcaataatcggcacaatcatacaaaggacgcgctgaagggccaatgatcccgctattatgaggcgcaacgtaccgccgggcactatcgctttaaacgcgggttgcggtaaagaataatgcgccgcgcaggcttcggtggtgattatccgcaaatgattatggttcgtaacgcggcaacatgctcaacagtcatgccaatggtgataatattgttgaatataagacctggtctgccaccgctgcggcaatcgctttttctcggtttgcgaaacctcgctgctcgaacgccgtattaacgacactggaagcccgacccgcgccaccgtgatggcgcgtaatcagaactgccgctcatggtgaatatccccagcggaccgtctgcgtggagacatccaacgaatttgccaacaatatcataaatataccacgctcgacacgatcaacactggtggtcgtgccgcgggttaccggttagttcagtgggctgtgaaaaattcctcgaaaaccatcaccctggcattttgccaaaaggtgacaaaaagatcgggtttgatcggtcactggggatcccgaagcaaatcccgccggatgatgtcgtttgcccgctacccgctggcgaagcggactgactcgcttcatcccaccacttgttgccagcgccaccgccaaagcgccgtgaaaacatcacccgcagtacatcaccaccacctcggctttgaaggccggttgatgctggcgcccaccaccagtagtcgcagcctgcacgctaccctgggtcataggcatgacaaatttagccaggcgacatgcctgttttggcgctgtctcttttcgcccgttaagcgcgccagacccggttctgaggccgcgcgatcgcgaaacgctactacccggctcacgccgatatcctgcggcgtaatccccgtccagaacaggtcatcaccgcctgacggtggggtgaagaacttttagcgccgtctgccagcgtacgtctgccagcacaacatcccgcaggaaatcgatttcctcaaccgcctctgcatcatcaggcagcagatccgggctggggtggttaatgattatccgctctgctagcggtatccgcatgatggccggattgccgaagatttcgcctggttataccgtttggtgtaacgggtgttaacgcccaggattccagctctgccagcaggctgttgccgatgtctgtcatcacctacgtatgcatcgaccctgcgcccacaacctttacccgccaccaaccgctaccgtcgccgctggcctgcaacttccgtataatttctcgccacatgcccaccgctctcgtcgtgtccttccacgtaatagatgcgatcctgtccacgtttatacctacacaagcagatcatggtcattctccttaaacattgcgggatgcgttcattttaattcaccagtgtttaaaagtgacggctacatcaattttgactgtcgatacaaaccagtcaaacgaacaaagcaaagcatgtcataaatgacaaaaagtgacataactgtattcaggagggttatggcaacaatcaccgacctcgttttacggacaatgggtccgccaatggcgagcaatttattgcagcaagaacgtaacttcgcgtcttgatgtgaacgccgaagctgccgacatctggtgaacaaggtgcgactcgccgccaaccggcgcagaccactaaagatgaatttatcattactgttcttgaatggcgatctggtgcgcaacattgttctgattgaaaacggcgtttgcgaaggcttatctgttcgctggtcgttgatatgtccacctcatgcaaaccgataaattcgttgccgatatacagcaaaggcttcagcatgatggatgttccgacgaaaccgtacttctgcaaatgccattaccggtactctgttactgctgatggcggcctgaaccgttgaacgatgccacgcccgtcccaccggtggcgatgggcggtggttgatcgcgctggcggtccgggcatggggatcacgttagctcatcagcaactacatgagcatcgcgctcaatgcgctctgacggaaaccgccgtttgtgaccctggatcttccgtgttgccgcaaagtgatgagcgcacgccgcaagtaagatcttcaccgcttcggcaaacaagtctcggcggagatcttctccgccatactcatgatcgatcttgccgcagaatcccagcatcgccttgatgtcgccaaccaaagctgcatcgtgccaatgctggggccgcctcgcagggttgtaactgagcgcgcggcgatcgcgatcgccaggacggtccgccattctggagcaggtcgtgtcaggtctgggatggctaccagtaaaaatgtaacgactggataaaggaataaatgaatgaataagtacaccatcaacgacattacgcgcgcatcgggcggttttgccatactggcggtcgatcagcaagccatgccgcaatgtttaccacagctggggcacctgctcggtagccgtgggcacaacgatttcaaagttaacactgcaaggccctctcgccttgtcctcggcgattctggtagatcagcaattcgccaccgccaggtggttgagcaaacgcgttatagcaggacgcgccatgattgtcatgccgatgagttcattctacagcagcagtattccggtcgatagcatggtgtcgaccgcaaaatcaatcgctacagatcaaacaagacggtggcaagcggcaaaactgctggtgctgtggcgtgatgaagatgcgcagcagcgtctggatatggtgaagagttcggcgaactgtgccactcacacggtgttgagccagtcattccgcccaccgcgtcgtggcgataaattcgatcgcgaacaagcgatcatcgataccgccagagctgggcgacggtggcgctgacctctcaaagttgaaatgccgctttatggcaggtccgcaacagaacttctgcttcacaacgtcagaccgagccacatcaatatgccatgcgggtgatctctcttccggtgtctcgtaagctgttcccgcattgccgtacgcgtggcaatgacggcgggcgcatcggacctggcaggccgtgcggtctgggcatcggtcgtcggtttaccagacaacgagctgatgctgcgtgacgtttgcaccgaagtacaacaacagcgacatcgtcagcaaaccaatggctaaacgccgctatgaatgaggataaagatggtttaacacctaagcttacaaccgttggctggaacggaaaccgaccatctttgattttggtaaaaattccgtagtgccgactggtttggctggttaggcaataaaggcaaatcaaagagatgggcaccatctgtggatcaccgctcattgcgtttattccgttgccacggcgtgggtcgacctggcgcttactcgttggttgatcacggtatcaagccatgagcgtgataaatatggcggctgagccatgcctgcacgtgaatgacggggcgtggtggatgcctcgagcagatatcaacgctaacagcatgccagcacgggtgcctgccagcgccgtcacggcagattttccaggcgctcgttacaccattgaaattatccagaaatatttctgaacgaagaaggcagatgtgctggagtcctgggacgaagccttccagcaaaaccgaagagtaccgcgacggcaatgccatatgcacgcggtggaaacttctcttgattgtttatgacgtcactcacgacaaaaatgagctggatcgcgcgattcgcgtggcttccccgcgatatccggcaatcgccgaaataatcattatcgcgttaacgaacacttcgatacccgtggaatccgctgccggattacaacaaagatcgccggcacgtcgcttccgcgcgttcgggtacaccaggccactggatcgaatggggccgtttaatgctgcacatcatgctgcctggaagcccgttgcgaacaaccagcgtaacgctgaagataccaaggtctgtttaacgccaccgtgcgcgatgcctgggcacccgatggcgcggacgggattgcgacataccgttgactgggaaggaaaaccggtggtccgcgaacgatgtacgttggcctatcaagcaatggtacggcctacgcgctccaccgtcactggcgatcgccagtatgaaaccctggtatcaaacatggtggggtgcattgagtacctgatggactatgaaaatggttcctggtggcggagctggatgcagttaatggtcctacaaagtctgggacgctaaacaggatattatcacctgctgcattgcctgagtgatcccacgtatcccgttagcgcccggcatgctccagcagtttgcagcagattactggataataatgcgaaataactgatctgaaaataggtgcgggtttcctctaaccctctccccaaaggggcgaggggacgtccggtgcagaaggttaaacgcaagcagacgccgaagatagagcattgagcaaggaacactctcgtttggaacatctggcaaacgcgaagcagacgccagcaatacgtaac

SEQ ID NO: 12 - DNA, 61 bp, Artificial Sequence
  Adapter design A/B (top strand)
  misc_binding (1)..(1): nucleotides preceded by 1x 5SpC3 and 29x iSpC3
  misc_binding (33)..(34): nucleotides separated by 1x iSp18
ggcgtctgcttgggtgtttaaccttttttttttaatgtacttcgttcagttacgtattgct

SEQ ID NO: 13 - DNA, 40 bp, Artificial Sequence
  Adapter design A (blocker strand)
  modified_base (1)..(1): 5BNA-G
  modified_base (2)..(2): iBNA-G
  modified_base (3)..(3): iBNA-T
  modified_base (4)..(4): iBNA-T
  modified_base (5)..(5): iBNA-A
ggttaaacacccaagcagacgcctaagtcagagaggttcc

SEQ ID NO: 14 - DNA, 45 bp, Artificial Sequence
  Adapter design A (bottom strand)
  modified_base (23)..(23): iBNA-A
  modified_base (24)..(24): iBNA-meC
  modified_base (25)..(25): iBNA-A
  modified_base (26)..(26): iBNA-T
  modified_base (27)..(27): iBNA-T
gcaatacgtaactgaacgaagtacatttttgaggcgagcggtcaa

SEQ ID NO: 15 - DNA, 41 bp, Artificial Sequence
  Adapter design B (blocker strand)
ggttaaacacccaagcagacgcctttgaggcgagcggtcaa

SEQ ID NO: 16 - DNA, 47 bp, Artificial Sequence
  Adapter design B (bottom strand)
  modified_base (23)..(23): iBNA-A
  modified_base (24)..(24): iBNA-meC
  modified_base (25)..(25): iBNA-A
  modified_base (26)..(26): iBNA-T
  modified_base (27)..(27): iBNA-T
gcaatacgtaactgaacgaagtacattttttaagtcagagaggttcc

SEQ ID NO: 17 - DNA, 80 bp, Artificial Sequence
  follow-on adapter top strand
  misc_binding (44)..(45): nucleotides separated by 4x iSp18
taacgaggttgtttctatctcggcgtctgcttgggtgtttaacctttttgtcagagaggttccaagtcagagaggttcct

SEQ ID NO: 18 - DNA, 123 bp, Artificial Sequence
  follow-on adapter bottom strand
  misc_binding (35)..(36): nucletoides separated by 4x iSp18
  misc_binding (98)..(99): nucletoides separated by 4x iSp18
ggaacctctctgacttggaacctctctgacaaaaaggttaaacacccaagcagacgccgagatagaaacaacccatcagattgtgtttgttagtcgctagcgactaacaaacacaatctgatg

SEQ ID NO: 19 - DNA, 70 bp, Artificial Sequence
  concatenation sequencing adapter top strand
  misc_binding (15)..(16): nucleotides separated by 15x iSpC3
  misc_binding (48)..(49): nucleotides separated by 1x iSp18
ggttgtttctatctcggcgtctgcttgggtgtttaaccttttttttttaatgtacttcgttcagttacgt

SEQ ID NO: 20 - DNA, 41 bp, Artificial Sequence; identical to SEQ ID NO: 15
  concatenation sequencing adapter blocker strand

SEQ ID NO: 21 - DNA, 28 bp, Artificial Sequence
  concatenation sequencing adapter bottom strand
  modified_base (24)..(24): iBNA-A
  modified_base (25)..(25): iBNA-meC
  modified_base (26)..(26): iBNA-A
  modified_base (27)..(27): iBNA-T
  modified_base (28)..(28): iBNA-T
tcgttaacgtaactgaacgaagtacatt

SEQ ID NO: 22 - DNA, 71 bp, Artificial Sequence
  fishing adapter top strand
  misc_binding (1)..(1): nucleotides preceded by 1 x 5SpC3 and 14 x iSpC3
  misc_binding (16)..(17): nucleotides separated by 15 x iSpC3
  misc_binding (49)..(50): nucleotides separated by 1 x iSp18
ttgtcagagaggttccggcgtctgcttgggtgtttaaccttttttttttaatgtacttcgttcagttacgt

SEQ ID NO: 23 - DNA, 22 bp, Artificial Sequence
  fishing adapter bottom strand
  modified_base (18)..(18): iBNA-A
  modified_base (19)..(19): iBNA-meC
  modified_base (20)..(20): iBNA-A
  modified_base (21)..(21): iBNA-T
  modified_base (22)..(22): iBNA-T
acgtaactgaacgaagtacatt

SEQ ID NO: 24 - DNA, 100 bp, Artificial Sequence
  fishing tether top strand
ttgtcagagaggttccttttttttttttttttttttttttttttttttttttttggttgtttctgttggtgctgatattgcttttttgaccgctcgcctc

SEQ ID NO: 25 - DNA, 31 bp, Artificial Sequence
  fishing tether bottom strand
  misc_binding (29)..(30): nucleotides separated by 6x iSp18
gcaatatcagcaccaacagaaacaacctttt

SEQ ID NO: 26 - DNA, 3587 bp, Artificial Sequence
  3.6kb dA-tailed DNA
gccatcagattgtgtttgttagtcgctgccatcagattgtgtttgttagtcgctttttttttttggaattttttttttggaattttttttttgcgctaacaacctcctgccgttttgcccgtgcatatcggtcacgaacaaatctgattactaaacacagtagcctggatttgttctatcagtaatcgaccttattcctaattaaatagagcaaatccccttattgggggtaagacatgaagatgccagaaaaacatgacctgttggccgccattctcgcggcaaaggaacaaggcatcggggcaatccttgcgtttgcaatggcgtaccttcgcggcagatataatggcggtgcgtttacaaaaacagtaatcgacgcaacgatgtgcgccattatcgcctagttcattcgtgaccttctcgacttcgccggactaagtagcaatctcgcttatataacgagcgtgtttatcggctacatcggtactgactcgattggttcgcttatcaaacgcttcgctgctaaaaaagccggagtagaagatggtagaaatcaataatcaacgtaaggcgttcctcgatatgctggcgtggtcggagggaactgataacggacgtcagaaaaccagaaatcatggttatgacgtcattgtaggcggagagctatttactgattactccgatcaccctcgcaaacttgtcacgctaaacccaaaactcaaatcaacaggcgccggacgctaccagcttctttcccgttggtgggatgcctaccgcaagcagcttggcctgaaagacttctctccgaaaagtcaggacgctgtggcattgcagcagattaaggagcgtggcgctttacctatgattgatcgtggtgatatccgtcaggcaatcgaccgttgcagcaatatctgggcttcactgccgggcgctggttatggtcagttcgagcataaggctgacagcctgattgcaaaattcaaagaagcgggcggaacggtcagagagattgatgtatgagcagagtcaccgcgattatctccgctctggttatctgcatcatcgtctgcctgtcatgggctgttaatcattaccgtgataacgccattacctacaaagcccagcgcgacaaaaatgccagagaactgaagctggcgaacgcggcaattactgacatgcagatgcgtcagcgtgatgttgctgcgctcgatgcaaaatacacgaaggagttagctgatgctaaagctgaaaatgatgctctgcgtgatgatgttgccgctggtcgtcgtcggttgcacatcaaagcagtctgtcagtcagtgcgtgaagccaccaccgcctccggcgtggataatgcagcctccccccgactggcagacaccgctgaacgggattatttcaccctcagagagaggctgatcactatgcaaaaacaactggaaggaacccagaagtatattaatgagcagtgcagatagagttgcccatatcgatgggcaactcatgcaattattgtgagcaatacacacgcgcttccagcggagtataaatgcctaaagtaataaaaccgagcaatccatttacgaatgtttgctgggtttctgttttaacaacattttctgcgccgccacaaattttggctgcatcgacagttttcttctgcccaattccagaaacgaagaaatgatgggtgatggtttcctttggtgctactgctgccggtttgttttgaacagtaaacgtctgttgagcacatcctgtaataagcagggccagcgcagtagcgagtagcatttttttcatggtgttattcccgatgctttttgaagttcgcagaatcgtatgtgtagaaaattaaacaaaccctaaacaatgagttgaaatttcatattgttaatatttattaatgtatgtcaggtgcgatgaatcgtcattgtattcccggattaactatgtccacagccctgacggggaacttctctgcgggagtgtccgggaataattaaaacgatgcacacagggtttagcgcgtacacgtattgcattatgccaacgccccggtgctgacacggaagaaaccggacgttatgatttagcgtggaaagatttgtgtagtgttctgaatgctctcagtaaatagtaatgaattatcaaaggtatagtaatatcttttatgttcatggatatttgtaacccatcggaaaactcctgctttagcaagattttccctgtattgctgaaatgtgatttctcttgatttcaacctatcataggacgtttctataagatgcgtgtttcttgagaatttaacatttacaacctttttaagtccttttattaacacggtgttatcgttttctaacacgatgtgaatattatctgtggctagatagtaaatataatgtgagacgttgtgacgttttagttcagaataaaacaattcacagtctaaatcttttcgcacttgatcgaatatttctttaaaaatggcaacctgagccattggtaaaaccttccatgtgatacgagggcgcgtagtttgcattatcgtttttatcgtttcaatctggtctgacctccttgtgttttgttgatgatttatgtcaaatattaggaatgttttcacttaatagtattggttgcgtaacaaagtgcggtcctgctggcattctggagggaaatacaaccgacagatgtatgtaaggccaacgtgctcaaatcttcatacagaaagatttgaagtaatattttaaccgctagatgaagagcaagcgcatggagcgacaaaatgaataaagaacaatctgctgatgatccctccgtggatctgattcgtgtaaaaaatatgcttaatagcaccatttctatgagttaccctgatgttgtaattgcatgtatagaacataaggtgtctctggaagcattcagagcaattgaggcagcgttggtgaagcacgataataatatgaaggattattccctggtggttgactgatcaccataactgctaatcattcaaactatttagtctgtgacagagccaacacgcagtctgtcactgtcaggaaagtggtaaaactgcaactcaattactgcaatgccctcgtaattaagtgaatttacaatatcgtcctgttcggagggaagaacgcgggatgttcattcttcatcacttttaattgatgtatatgctctcttttctgacgttagtctccgacggcaggcttcaatgacccaggctgagaaattcccggaccctttttgctcaagagcgatgttaatttgttcaatcatttggttaggaaagcggatgttgcgggttgttgttctgcgggttctgttcttcgttgacatgaggttgccccgtattcagtgtcgctgatttgtattgtctgaagttgtttttacgttaagttgatgcagatcaattaatacgatacctgcgtcataattgattatttgacgtggtttgatggcctccacgcacgttgtgatatgtagatgataatcattatcactttacgggtcctttccggtgaaaaaaaaggtaccaaaaaaaacatcgtcgtgagtagtgaaccgtaagc

SEQ ID NO: 27 - DNA, 41 bp, Artificial Sequence
  follow-on adapter bottom strand
acgtaactgaacgaagtacatttttgaggccgagcggtcaa

SEQ ID NO: 28 - DNA, 40 bp, Artificial Sequence; identical to SEQ ID NO: 13
  follow-on adapter blocker strand

SEQ ID NO: 29 - DNA, 38 bp, Artificial Sequence
  FO016_FOSEN_tailattach_TOP_A
ggtgctgaagaaagttgtcggtgtctttgtgttaacct

SEQ ID NO: 30 - DNA, 60 bp, Artificial Sequence
  FO017_FOSEN_tailattach_BOT_A
ggttaacacaaagacaccgacaactttcttcagcaccagcaattaagtcagagaggttcc

SEQ ID NO: 31 - DNA, 77 bp, Artificial Sequence
  FO018_FOSEN_tailattach_TOP_B
  misc_binding (23)..(24): nucleotides separated by 4x iSp18
ccaatttgtgggttcgtctgcggtttttggcgtctgcttgggtgtttaaccaaggcgtctgcttgggtgtttaacct

SEQ ID NO: 32 - DNA, 99 bp, Artificial Sequence
  FO019_FOSEN_tailattach_BOT_B
  misc_binding (53)..(54): nucleotides separated by iSp18
ggttaaacacccaagcagacgccttggttaaacacccaagcagacgccaaaaaccgcagacgaacccacaaattggagcaattaagtcagagaggttcc

SEQ ID NO: 33 - DNA, 82 bp, Artificial Sequence
  FO020_FOSEN_tailattach_BOT_B_noside
  misc_binding (53)..(54): nucleotides separated by 4x iSp18
ggttaaacacccaagcagacgccttggttaaacacccaagcagacgccaaaaaccgcagacgaacccacaaattggagcaat

SEQ ID NO: 34 - DNA, 66 bp, Artificial Sequence
  FO021_FOSEN_tailattach_TOP_C
  misc_binding (23)..(24): nucleoitdes separated by 4x iSp18
  misc_binding (23)..(24): nucleotides separated by 4x iSp18
ggcgtctgcttgggtgtttaacctttttggtgctgaagaaagttgtcggtgtctttgtgttaacct

SEQ ID NO: 35 - DNA, 88 bp, Artificial Sequence
  FO022_FOSEN_tailattach_BOT_C
  misc_binding (42)..(43): nucleotides separated by 4x iSp18
ggttaacacaaagacaccgacaactttcttcagcaccaaaaaggttaaacacccaagcagacgccagcaattaagtcagagaggttcc

SEQ ID NO: 36 - DNA, 44 bp, Artificial Sequence
  FO023_FOSEN_splintagain_TOP_A
  misc_binding (15)..(16): nucleotides separated by 4x iSp18
ccaatttgtggttcctttttggcgtctgcttgggtgtttaacct

SEQ ID NO: 37 - DNA, 49 bp, Artificial Sequence
  FO024_FOSEN_splintagain_BOT_A
  misc_binding (28)..(29): nucleotides separated by 4x iSp18
ggttaaacacccaagcagacgccaaaaaggaaccacaaattggagcaat

SEQ ID NO: 38 - DNA, 69 bp, Artificial Sequence
  FO025_FOSEN_splintagain_TOP_B
  misc_binding (15)..(16): nucleotides separated by 4x iSp18
ccaatttgtggttcctttttggcgtctgcttgggtgtttaaccaaggcgtctgcttgggtgtttaacct

SEQ ID NO: 39 - DNA, 74 bp, Artificial Sequence
  FO026_FOSEN_splintagain_BOT_B
  misc_binding (53)..(54): nucleotides separeted by 4x iSp18
ggttaaacacccaagcagacgccttggttaaacacccaagcagacgccaaaaaggaaccacaaattggagcaat

SEQ ID NO: 40 - DNA, 61 bp, Artificial Sequence
  FO027_TOP_1sp18
  misc_binding (23)..(24): nucleotides separated by 1x iSp18
ggcgtctgcttgggtgtttaacctttttgtcagagaggttccaagtcagagaggttccaat

SEQ ID NO: 41 - DNA, 66 bp, Artificial Sequence
  FO028_BOT_1sp18
  misc_binding (37)..(38): nucleotides separated by 1x iSp18
ttggaacctctctgacttggaacctctctgacaaaaaggttaaacacccaagcagacgccagcaat

SEQ ID NO: 42 - DNA, 45 bp, Artificial Sequence
  FO029_TOP_1hybsite
  misc_binding (23)..(24): nucleotides separated by 4x iSp18
ggcgtctgcttgggtgtttaacctttttgtcagagaggttccaat

SEQ ID NO: 43 - DNA, 50 bp, Artificial Sequence
  FO030_BOT_1hybsite
  misc_binding (21)..(22): nucleotides separated by 4x iSp18
ttggaacctctctgacaaaaaggttaaacacccaagcagacgccagcaat

SEQ ID NO: 44 - DNA, 40 bp, Artificial Sequence; identical to SEQ ID NO: 13
  Blocker strand ID2 (TT008)

SEQ ID NO: 45 - DNA, 14 bp, Artificial Sequence
  Pore-tether
ggaacctctctgac

SEQ ID NO: 46 - DNA, 47 bp, Artificial Sequence; identical to SEQ ID NO: 16
  Bottom strand ID5 (TT186)